European Patent Application EP 4 159 237 A1, published April 5, 2023. Title: Improved granzyme B variants. Applicant: CHUGAI SEIYAKU KABUSHIKI KAISHA. The sequence listing filed with the application follows.

SEQUENCE LISTING (17 sequences)

SEQ ID NO: 1 - protein, 247 aa, Homo sapiens
MQPILLLLAFLLLPRADAGEIIGGHEAKPHSRPYMAYLMIWDQKSLKRCGGFLIRDDFVLTAAHCWGSSINVTLGAHNIKEQEPTQQFIPVKRPIPHPAYNPKNFSNDIMLLQLERKAKRTRAVQPLRLPSNKAQVKPGQTCSVAGWGQTAPLGKHSHTLQEVKMTVQEDRKCESDLRHYYDSTIELCVGDPEIKKTSFKGDSGGPLVCNKVAQGIVSYGRNNGMPPRACTKVSSFVHWIKKTMKRY

SEQ ID NO: 2 - protein, 227 aa, Homo sapiens
IIGGHEAKPHSRPYMAYLMIWDQKSLKRCGGFLIRDDFVLTAAHCWGSSINVTLGAHNIKEQEPTQQFIPVKRPIPHPAYNPKNFSNDIMLLQLERKAKRTRAVQPLRLPSNKAQVKPGQTCSVAGWGQTAPLGKHSHTLQEVKMTVQEDRKCESDLRHYYDSTIELCVGDPEIKKTSFKGDSGGPLVCNKVAQGIVSYGRNNGMPPRACTKVSSFVHWIKKTMKRY

SEQ ID NO: 3 - protein, 31 aa, Artificial Sequence
  An artificial signal sequence
MGILPSPGMPALLSLVSLLSVLLMGCVAETG

SEQ ID NO: 4 - protein, 5 aa, Artificial Sequence
  An enterokinase recognition sequence
DDDDK

SEQ ID NO: 5 - protein, 272 aa, Artificial Sequence
  An artificially synthesized peptide sequence
MGILPSPGMPALLSLVSLLSVLLMGCVAETGDDDDKIIGGHEAKPHSRPYMAYLMIWDQKSLKRCGGFLIRDDFVLTAAHCWGSSINVTLGAHNIKEQEPTQQFIPVKRPIPHPAYNPKNFSNDIMLLQLERKAKRTRAVQPLRLPSNKAQVKPGQTCSVAGWGQTAPLGKHSHTLQEVKMTVQEDRKCESDLRHYYDSTIELCVGDPEIKKTSFKGDSGGPLVCNKVAQGIVSYGRNNGMPPRACTKVSSFVHWIKKTMKRYGTKHHHHHH

SEQ ID NO: 6 - protein, 227 aa, Artificial Sequence
  An artificially synthesized peptide sequence
IIGGHEAKPHSRPYMAYLMIWDQLSLKKCGGFLIRDDFVLTAAHCWGSSINVTLGAHNIKEQEPTQQFIPVKRPIPHPAYNPKNFSNDIMLLQLERKAKRTRAVQPLRLPSNKAQVKPGQTCSVAGWGQTAPLGPHSHTLQEVKMTVQEDRLCEIDLRHYYDSTIELCVGDPEIKKTSFRGDSGGPLVCNKVAQGIVSYGRNNGMPPRACTKVSSFVHWIKKTMKRY

SEQ ID NO: 7 - protein, 227 aa, Artificial Sequence
  An artificially synthesized peptide sequence
IIGGHEAKPHSRPYMAYLMIWDQLSLKECGGFLIRDDFVLTAAHCWGSSINVTLGAHNIKEQEPTQQFIPVKRPIPHPAYNPKNFSNDIMLLQLERKAKRTRAVQPLRLPSNKAQVKPGQTCSVAGWGQTAPLGPHSHTLQEVKMTVQEDRLCEIDLRHYYDSTIELCVGDPEIKKTSFRGDSGGPLVCNKVAQGIVSYGRNNGMPPRACTKVSSFVHWIKKTMKRY

SEQ ID NO: 8 - protein, 227 aa, Artificial Sequence
  An artificially synthesized peptide sequence
IIGGHEAKPHSRPYMAYLMIWDQFSLKKCGGFLIRDDFVLTAAHCWGSSINVTLGAHNIKEQEPTQQFIPVKRPIPHPAYNPKNFSNDIMLLQLERKAKRTRAVQPLRLPSNKAQVKPGQTCSVAGWGQTAPLGPHSHTLQEVKMTVQEDRLCEIDLRHYYDSTIELCVGDPEIKKTSFRGDSGGPLVCNKVAQGIVSYGRNNGMPPRACTKVSSFVHWIKKTMKRY

SEQ ID NO: 9 - protein, 227 aa, Artificial Sequence
  An artificially synthesized peptide sequence
IIGGHEAKPHSRPYMAYLMIWDQFSLKECGGFLIRDDFVLTAAHCWGSSINVTLGAHNIKEQEPTQQFIPVKRPIPHPAYNPKNFSNDIMLLQLERKAKRTRAVQPLRLPSNKAQVKPGQTCSVAGWGQTAPLGPHSHTLQEVKMTVQEDRLCEIDLRHYYDSTIELCVGDPEIKKTSFRGDSGGPLVCNKVAQGIVSYGRNNGMPPRACTKVSSFVHWIKKTMKRY

SEQ ID NO: 10 - protein, 227 aa, Artificial Sequence
  An artificially synthesized peptide sequence
IIGGHEAKPHSRPYMAYLMIWDQLSIKRCGGFLIRDDFVLTAAHCWGSSINVTLGAHNIKEQEPTQQFIPVKRPIPHPAYNPKNFSNDIMLLQLERKAKRTRAVQPLRLPSNKAQVKPGQTCSVAGWGQTAPLGPHSHTLQEVKMTVQEDRLCEIDLRHYYDSTIELCVGDPEIKKTSFRGDSGGPLVCNKVAQGIVSYGRNNGMPPRACTKVSSFVHWIKKTMKRY

SEQ ID NO: 11 - protein, 227 aa, Artificial Sequence
  An artificially synthesized peptide sequence
IIGGHEAKPHSRPYMAYLMIWDQLSEKRCGGFLIRDDFVLTAAHCWGSSINVTLGAHNIKEQEPTQQFIPVKRPIPHPAYNPKNFSNDIMLLQLERKAKRTRAVQPLRLPSNKAQVKPGQTCSVAGWGQTAPLGPHSHTLQEVKMTVQEDRLCEIDLRHYYDSTIELCVGDPEIKKTSFRGDSGGPLVCNKVAQGIVSYGRNNGMPPRACTKVSSFVHWIKKTMKRY

SEQ ID NO: 12 - protein, 227 aa, Artificial Sequence
  An artificially synthesized peptide sequence
IIGGHEAKPHSRPYMAYLMIWDQLSFKRCGGFLIRDDFVLTAAHCWGSSINVTLGAHNIKEQEPTQQFIPVKRPIPHPAYNPKNFSNDIMLLQLERKAKRTRAVQPLRLPSNKAQVKPGQTCSVAGWGQTAPLGPHSHTLQEVKMTVQEDRLCEIDLRHYYDSTIELCVGDPEIKKTSFRGDSGGPLVCNKVAQGIVSYGRNNGMPPRACTKVSSFVHWIKKTMKRY

SEQ ID NO: 13 - protein, 227 aa, Artificial Sequence
  An artificially synthesized peptide sequence
IIGGHEAKPHSRPYMAYLMIWDQLSQKRCGGFLIRDDFVLTAAHCWGSSINVTLGAHNIKEQEPTQQFIPVKRPIPHPAYNPKNFSNDIMLLQLERKAKRTRAVQPLRLPSNKAQVKPGQTCSVAGWGQTAPLGPHSHTLQEVKMTVQEDRLCEIDLRHYYDSTIELCVGDPEIKKTSFRGDSGGPLVCNKVAQGIVSYGRNNGMPPRACTKVSSFVHWIKKTMKRY

SEQ ID NO: 14 - protein, 227 aa, Artificial Sequence
  An artificially synthesized peptide sequence
IIGGHEAKPHSRPYMAYLMIWDQFSIKRCGGFLIRDDFVLTAAHCWGSSINVTLGAHNIKEQEPTQQFIPVKRPIPHPAYNPKNFSNDIMLLQLERKAKRTRAVQPLRLPSNKAQVKPGQTCSVAGWGQTAPLGPHSHTLQEVKMTVQEDRLCEIDLRHYYDSTIELCVGDPEIKKTSFRGDSGGPLVCNKVAQGIVSYGRNNGMPPRACTKVSSFVHWIKKTMKRY

SEQ ID NO: 15 - protein, 227 aa, Artificial Sequence
  An artificially synthesized peptide sequence
IIGGHEAKPHSRPYMAYLMIWDQFSEKRCGGFLIRDDFVLTAAHCWGSSINVTLGAHNIKEQEPTQQFIPVKRPIPHPAYNPKNFSNDIMLLQLERKAKRTRAVQPLRLPSNKAQVKPGQTCSVAGWGQTAPLGPHSHTLQEVKMTVQEDRLCEIDLRHYYDSTIELCVGDPEIKKTSFRGDSGGPLVCNKVAQGIVSYGRNNGMPPRACTKVSSFVHWIKKTMKRY

SEQ ID NO: 16 - protein, 227 aa, Artificial Sequence
  An artificially synthesized peptide sequence
IIGGHEAKPHSRPYMAYLMIWDQFSFKRCGGFLIRDDFVLTAAHCWGSSINVTLGAHNIKEQEPTQQFIPVKRPIPHPAYNPKNFSNDIMLLQLERKAKRTRAVQPLRLPSNKAQVKPGQTCSVAGWGQTAPLGPHSHTLQEVKMTVQEDRLCEIDLRHYYDSTIELCVGDPEIKKTSFRGDSGGPLVCNKVAQGIVSYGRNNGMPPRACTKVSSFVHWIKKTMKRY

SEQ ID NO: 17 - protein, 227 aa, Artificial Sequence
  An artificially synthesized peptide sequence
IIGGHEAKPHSRPYMAYLMIWDQFSQKRCGGFLIRDDFVLTAAHCWGSSINVTLGAHNIKEQEPTQQFIPVKRPIPHPAYNPKNFSNDIMLLQLERKAKRTRAVQPLRLPSNKAQVKPGQTCSVAGWGQTAPLGPHSHTLQEVKMTVQEDRLCEIDLRHYYDSTIELCVGDPEIKKTSFRGDSGGPLVCNKVAQGIVSYGRNNGMPPRACTKVSSFVHWIKKTMKRY